European Patent Specification EP 3 160 994 B1, published February 19, 2025. Title: MULTISPECIFIC ANTIGEN BINDING PROTEINS. Applicant: INNATE PHARMA. The sequence listing filed with the application follows.

SEQUENCE LISTING (56 sequences)

SEQ ID NO: 1 - protein, 216 aa, Homo sapiens
APELLGGPSVFLFPPKPKDTLMISRTPEVTCVVVDVSHEDPEVKFNWYVDGVEVHNAKTKPREEQYNSTYRVVSVLTVLHQDWLNGKEYKCKVSNKALPAPIEKTISKAKGQPREPQVYTLPPSREEMTKNQVSLTCLVKGFYPSDIAVEWESNGQPENNYKTTPPVLDSDGSFFLTSKLTVDKSRWQQGNVFSCSVMHEALHNHYTQKSLSLSPG

SEQ ID NO: 2 - protein, 227 aa, Homo sapiens
GQPREPQVYTLPPSREEMTKNQVSLTCLVKGFYPSDIAVEWESNGQPENNYKTTPPVLDSDGSFFLYSKLTVDKSRWQQGNVFSCSVMHEALHNHYTQKSLSLSPGGGGGSGGGGSGGGGSGQPREPQVYTLPPSREEMTKNQVSLTCLVKGFYPSDIAVEWESNGQPENNYKTTPPVLDSDGSFFLYSKLTVDKSRWQQGNVFSCSVMHEALHNHYTQKSLSLSPG

SEQ ID NO: 3 - DNA, 333 bp, mus musculus
gacattcagctgacccaatctccagcttctttggctgtgtctctagggcagagggccaccatctcctgcaaggccagccaaagtgttgattatgatggtgatagttatttgaactggtaccaacagataccaggacagccacccaaactcctcatctatgatgcatccaatctagtatctgggattccacccaggtttagtggcagtgggtctgggacagacttcaccctcaacatccatcctgtggagaaggtggatgctgcaacctatcactgtcagcaaagtactgaggacccttggacgttcggtggaggcaccaagctggaaatcaaa

SEQ ID NO: 4 - protein, 111 aa, mus musculus
DIQLTQSPASLAVSLGQRATISCKASQSVDYDGDSYLNWYQQIPGQPPKLLIYDASNLVSGIPPRFSGSGSGTDFTLNIHPVEKVDAATYHCQQSTEDPWTFGGGTKLEIK

SEQ ID NO: 5 - DNA, 372 bp, mus musculus
caggttcagctgcagcagtctggggctgagctggtgcggcctgggtcctcagtgaagatttcctgcaaagcatctggctacgcattcagtagctactggatgaactgggtgaagcagaggcctggacagggtcttgagtggattggacagatttggcctggagatggtgatactaactacaacggaaagttcaagggcaaggccacactgactgcagacgaatcctccagcacagcctacatgcagctcagcagcctggcctctgaggactctgcggtctatttctgtgcaagacgagaaacgaccactgtcgggcgttattactatgctatggactactggggtcaaggaaccacagtcaccgtctcctca

SEQ ID NO: 6 - protein, 124 aa, mus musculus
QVQLQQSGAELVRPGSSVKISCKASGYAFSSYWMNWVKQRPGQGLEWIGQIWPGDGDTNYNGKFKGKATLTADESSSTAYMQLSSLASEDSAVYFCARRETTTVGRYYYAMDYWGQGTTVTVSS

SEQ ID NO: 7 - DNA, 648 bp, homo sapiens
gcacctgaactcctggggggaccgtcagtcttcctcttccccccaaaacccaaggacaccctcatgatctcccggacccctgaggtcacatgcgtggtggtggacgtgagccacgaagaccctgaggtcaagttcaactggtacgtggacggcgtggaggtgcataatgccaagacaaagccgcgggaggagcagtacaacagcacgtaccgtgtggtcagcgtcctcaccgtcctgcaccaggactggctgaatggcaaggagtacaagtgcaaggtctccaacaaagccctcccagcccccatcgagaaaaccatctccaaagccaaagggcagccccgagaaccacaggtgtacaccaagcccccatcccgggaggagatgaccaagaaccaggtcagcctgtcctgcctggtcaaaggcttctatcccagcgacatcgccgtggagtgggagagcaatgggcagccggagaacaactacaagaccacggttcccgtgctggactccgacggctccttccgcctcgctagctacctcaccgtggacaagagcaggtggcagcaggggaacgtcttctcatgctccgtgatgcatgaggctctgcacaaccactacacgcagaagagcctctccctgtccccgggg

SEQ ID NO: 8 - protein, 216 aa, homo sapiens
APELLGGPSVFLFPPKPKDTLMISRTPEVTCVVVDVSHEDPEVKFNWYVDGVEVHNAKTKPREEQYNSTYRVVSVLTVLHQDWLNGKEYKCKVSNKALPAPIEKTISKAKGQPREPQVYTKPPSREEMTKNQVSLSCLVKGFYPSDIAVEWESNGQPENNYKTTVPVLDSDGSFRLASYLTVDKSRWQQGNVFSCSVMHEALHNHYTQKSLSLSPG

SEQ ID NO: 9 - protein, 718 aa, Artificial
  Chimeric homo sapiens-mus musculus
DIQLTQSPASLAVSLGQRATISCKASQSVDYDGDSYLNWYQQIPGQPPKLLIYDASNLVSGIPPRFSGSGSGTDFTLNIHPVEKVDAATYHCQQSTEDPWTFGGGTKLEIKGGGGSGGGGSGGGGSQVQLQQSGAELVRPGSSVKISCKASGYAFSSYWMNWVKQRPGQGLEWIGQIWPGDGDTNYNGKFKGKATLTADESSSTAYMQLSSLASEDSAVYFCARRETTTVGRYYYAMDYWGQGTTVTVSSGGGSSAPELLGGPSVFLFPPKPKDTLMISRTPEVTCVVVDVSHEDPEVKFNWYVDGVEVHNAKTKPREEQYNSTYRVVSVLTVLHQDWLNGKEYKCKVSNKALPAPIEKTISKAKGQPREPQVYTKPPSREEMTKNQVSLSCLVKGFYPSDIAVEWESNGQPENNYKTTVPVLDSDGSFRLASYLTVDKSRWQQGNVFSCSVMHEALHNHYTQKSLSLSPGSTGSDIKLQQSGAELARPGASVKMSCKTSGYTFTRYTMHWVKQRPGQGLEWIGYINPSRGYTNYNQKFKDKATLTTDKSSSTAYMQLSSLTSEDSAVYYCARYYDDHYCLDYWGQGTTLTVSSVEGGSGGSGGSGGSGGVDDIQLTQSPAIMSASPGEKVTMTCRASSSVSYMNWYQQKSGTSPKRWIYDTSKVASGVPYRFSGSGSGTSYSLTISSMEAEDAATYYCQQWSSNPLTFGAGTKLELK

SEQ ID NO: 10 - protein, 245 aa, Mus musculus
STGSEVQLQQSGPELVKPGASVKISCKTSGYTFTEYTMHWVKQSHGKSLEWIGGISPNIGGTSYNQKFKGKATLTVDKSSSTAYMELRSLTSEDSAVYYCARRGGSFDYWGQGTTLTVSSVEGGSGGSGGSGGSGGVDDIVMTQSPATLSVTPGDRVSLSCRASQSISDYLHWYQQKSHESPRLLIKYASQSISGIPSRFSGSGSGSDFTLSINSVEPEDVGVYYCQNGHSFPLTFGAGTKLELK

SEQ ID NO: 11 - protein, 698 aa, Artificial
  Chimeric homo sapiens - mus musculus
DIQLTQSPASLAVSLGQRATISCKASQSVDYDGDSYLNWYQQIPGQPPKLLIYDASNLVSGIPPRFSGSGSGTDFTLNIHPVEKVDAATYHCQQSTEDPWTFGGGTKLEIKGGGGSGGGGSGGGGSQVQLQQSGAELVRPGSSVKISCKASGYAFSSYWMNWVKQRPGQGLEWIGQIWPGDGDTNYNGKFKGKATLTADESSSTAYMQLSSLASEDSAVYFCARRETTTVGRYYYAMDYWGQGTTVTVSSGGGSSAPELLGGPSVFLFPPKPKDTLMISRTPEVTCVVVDVSHEDPEVKFNWYVDGVEVHNAKTKPREEQYNSTYRVVSVLTVLHQDWLNGKEYKCKVSNKALPAPIEKTISKAKGQPREPQVYTKPPSREEMTKNQVSLSCLVKGFYPSDIAVEWESNGQPENNYKTTVPVLDSDGSFRLASYLTVDKSRWQQGNVFSCSVMHEALHNHYTQKSLSLSPGSTGSEVQLQQSGPELVKPGASVKISCKTSGYTFTEYTMHWVKQSHGKSLEWIGGISPNIGGTSYNQKFKGKATLTVDKSSSTAYMELRSLTSEDSAVYYCARRGGSFDYWGQGTTLTVSSASTKGPSVFPLAPSSKSTSGGTAALGCLVKDYFPEPVTVSWNSGALTSGVHTFPAVLQSSGLYSLSSVVTVPSSSLGTQTYICNVNHKPSNTKVDKRVEPKSCDKTH

SEQ ID NO: 12 - protein, 214 aa, Artificial
  Chimeric - homo sapiens mus musculus
DIVMTQSPATLSVTPGDRVSLSCRASQSISDYLHWYQQKSHESPRLLIKYASQSISGIPSRFSGSGSGSDFTLSINSVEPEDVGVYYCQNGHSFPLTFGAGTKLELKRTVAAPSVFIFPPSDEQLKSGTASVVCLLNNFYPREAKVQWKVDNALQSGNSQESVTEQDSKDSTYSLSSTLTLSKADYEKHKVYACEVTHQGLSSPVTKSFNRGEC

SEQ ID NO: 13 - protein, 218 aa, Artificial
  Chimeric homo sapiens mus musculus
DIQLTQSPASLAVSLGQRATISCKASQSVDYDGDSYLNWYQQIPGQPPKLLIYDASNLVSGIPPRFSGSGSGTDFTLNIHPVEKVDAATYHCQQSTEDPWTFGGGTKLEIKRTVAAPSVFIFPPSDEQLKSGTASVVCLLNNFYPREAKVQWKVDNALQSGNSQESVTEQDSKDSTYSLSSTLTLSKADYEKHKVYACEVTHQGLSSPVTKSFNRGEC

SEQ ID NO: 14 - protein, 675 aa, Artificial
  Chimeric homo sapiens mus musculus
QVQLQQSGAELVRPGSSVKISCKASGYAFSSYWMNWVKQRPGQGLEWIGQIWPGDGDTNYNGKFKGKATLTADESSSTAYMQLSSLASEDSAVYFCARRETTTVGRYYYAMDYWGQGTTVTVSSASTKGPSVFPLAPSSKSTSGGTAALGCLVKDYFPEPVTVSWNSGALTSGVHTFPAVLQSSGLYSLSSVVTVPSSSLGTQTYICNVNHKPSNTKVDKRVEPKSCGGGSSAPELLGGPSVFLFPPKPKDTLMISRTPEVTCVVVDVSHEDPEVKFNWYVDGVEVHNAKTKPREEQYSSTYRVVSVLTVLHQDWLNGKEYKCKVSNKALPAPIEKTISKAKGQPREPQVYTKPPSREEMTKNQVSLSCLVKGFYPSDIAVEWESNGQPENNYKTTVPVLDSDGSFRLASYLTVDKSRWQQGNVFSCSVMHEALHNHYTQKSLSLSPGSTGSEVQLQQSGPELVKPGASVKISCKTSGYTFTEYTMHWVKQSHGKSLEWIGGISPNIGGTSYNQKFKGKATLTVDKSSSTAYMELRSLTSEDSAVYYCARRGGSFDYWGQGTTLTVSSRTVAAPSVFIFPPSDEQLKSGTASVVCLLNNFYPREAKVQWKVDNALQSGNSQESVTEQDSKDSTYSLSSTLTLSKADYEKHKVYACEVTHQGLSSPVTKSFNRGEC

SEQ ID NO: 15 - protein, 214 aa, Artificial
  Chimeric homo sapiens mus musculus
DIVMTQSPATLSVTPGDRVSLSCRASQSISDYLHWYQQKSHESPRLLIKYASQSISGIPSRFSGSGSGSDFTLSINSVEPEDVGVYYCQNGHSFPLTFGAGTKLELKASTKGPSVFPLAPSSKSTSGGTAALGCLVKDYFPEPVTVSWNSGALTSGVHTFPAVLQSSGLYSLSSVVTVPSSSLGTQTYICNVNHKPSNTKVDKRVEPKSCDKTH

SEQ ID NO: 16 - protein, 218 aa, Artificial; identical to SEQ ID NO: 13
  Chimeric homo sapiens mus musculus

SEQ ID NO: 17 - protein, 801 aa, Artificial
  Chimeric homo sapiens mus musculus
QVQLQQSGAELVRPGSSVKISCKASGYAFSSYWMNWVKQRPGQGLEWIGQIWPGDGDTNYNGKFKGKATLTADESSSTAYMQLSSLASEDSAVYFCARRETTTVGRYYYAMDYWGQGTTVTVSSASTKGPSVFPLAPSSKSTSGGTAALGCLVKDYFPEPVTVSWNSGALTSGVHTFPAVLQSSGLYSLSSVVTVPSSSLGTQTYICNVNHKPSNTKVDKRVEPKSCDKTHTCPPCPAPELLGGPSVFLFPPKPKDTLMISRTPEVTCVVVDVSHEDPEVKFNWYVDGVEVHNAKTKPREEQYSSTYRVVSVLTVLHQDWLNGKEYKCKVSNKALPAPIEKTISKAKGQPREPQVYTLPPSREEMTKNQVSLTCLVKGFYPSDIAVEWESNGQPENNYKTTPPVLDSDGSFFLYSKLTVDKSRWQQGNVFSCSVMHEALHNHYTQKSLSLSPGGGGGSGGGGSGGGGSGQPREPQVYTLPPSREEMTKNQVSLTCLVKGFYPSDIAVEWESNGQPENNYKTTPPVLDSDGSFFLYSKLTVDKSRWQQGNVFSCSVMHEALHNHYTQKSLSLSPGSTGSEVQLQQSGPELVKPGASVKISCKTSGYTFTEYTMHWVKQSHGKSLEWIGGISPNIGGTSYNQKFKGKATLTVDKSSSTAYMELRSLTSEDSAVYYCARRGGSFDYWGQGTTLTVSSRTVAAPSVFIFPPSDEQLKSGTASVVCLLNNFYPREAKVQWKVDNALQSGNSQESVTEQDSKDSTYSLSSTLTLSKADYEKHKVYACEVTHQGLSSPVTKSFNRGEC

SEQ ID NO: 18 - protein, 214 aa, Artificial; identical to SEQ ID NO: 15
  Chimeric homo sapiens mus musculus

SEQ ID NO: 19 - protein, 218 aa, Artificial; identical to SEQ ID NO: 13
  Chimeric homo sapiens mus musculus

SEQ ID NO: 20 - protein, 801 aa, Artificial
  Chimeric homo sapiens mus musculus
QVQLQQSGAELVRPGSSVKISCKASGYAFSSYWMNWVKQRPGQGLEWIGQIWPGDGDTNYNGKFKGKATLTADESSSTAYMQLSSLASEDSAVYFCARRETTTVGRYYYAMDYWGQGTTVTVSSASTKGPSVFPLAPSSKSTSGGTAALGCLVKDYFPEPVTVSWNSGALTSGVHTFPAVLQSSGLYSLSSVVTVPSSSLGTQTYICNVNHKPSNTKVDKRVEPKSCDKTHTSPPSPAPELLGGPSVFLFPPKPKDTLMISRTPEVTCVVVDVSHEDPEVKFNWYVDGVEVHNAKTKPREEQYSSTYRVVSVLTVLHQDWLNGKEYKCKVSNKALPAPIEKTISKAKGQPREPQVYTLPPSREEMTKNQVSLTCLVKGFYPSDIAVEWESNGQPENNYKTTPPVLDSDGSFFLYSKLTVDKSRWQQGNVFSCSVMHEALHNHYTQKSLSLSPGGGGGSGGGGSGGGGSGQPREPQVYTLPPSREEMTKNQVSLTCLVKGFYPSDIAVEWESNGQPENNYKTTPPVLDSDGSFFLYSKLTVDKSRWQQGNVFSCSVMHEALHNHYTQKSLSLSPGSTGSEVQLQQSGPELVKPGASVKISCKTSGYTFTEYTMHWVKQSHGKSLEWIGGISPNIGGTSYNQKFKGKATLTVDKSSSTAYMELRSLTSEDSAVYYCARRGGSFDYWGQGTTLTVSSRTVAAPSVFIFPPSDEQLKSGTASVVCLLNNFYPREAKVQWKVDNALQSGNSQESVTEQDSKDSTYSLSSTLTLSKADYEKHKVYACEVTHQGLSSPVTKSFNRGEC

SEQ ID NO: 21 - protein, 214 aa, Artificial; identical to SEQ ID NO: 15
  Chimeric homo sapiens mus musculus

SEQ ID NO: 22 - protein, 218 aa, Artificial; identical to SEQ ID NO: 13
  Chimeric homo sapiens mus musculus

SEQ ID NO: 23 - protein, 796 aa, Artificial
  Chimeric homo sapiens mus musculus
QVQLQQSGAELVRPGSSVKISCKASGYAFSSYWMNWVKQRPGQGLEWIGQIWPGDGDTNYNGKFKGKATLTADESSSTAYMQLSSLASEDSAVYFCARRETTTVGRYYYAMDYWGQGTTVTVSSASTKGPSVFPLAPSSKSTSGGTAALGCLVKDYFPEPVTVSWNSGALTSGVHTFPAVLQSSGLYSLSSVVTVPSSSLGTQTYICNVNHKPSNTKVDKRVEPKSCGGGSSAPELLGGPSVFLFPPKPKDTLMISRTPEVTCVVVDVSHEDPEVKFNWYVDGVEVHNAKTKPREEQYSSTYRVVSVLTVLHQDWLNGKEYKCKVSNKALPAPIEKTISKAKGQPREPQVYTLPPSREEMTKNQVSLTCLVKGFYPSDIAVEWESNGQPENNYKTTPPVLDSDGSFFLYSKLTVDKSRWQQGNVFSCSVMHEALHNHYTQKSLSLSPGGGGGSGGGGSGGGGSGQPREPQVYTLPPSREEMTKNQVSLTCLVKGFYPSDIAVEWESNGQPENNYKTTPPVLDSDGSFFLYSKLTVDKSRWQQGNVFSCSVMHEALHNHYTQKSLSLSPGSTGSEVQLQQSGPELVKPGASVKISCKTSGYTFTEYTMHWVKQSHGKSLEWIGGISPNIGGTSYNQKFKGKATLTVDKSSSTAYMELRSLTSEDSAVYYCARRGGSFDYWGQGTTLTVSSRTVAAPSVFIFPPSDEQLKSGTASVVCLLNNFYPREAKVQWKVDNALQSGNSQESVTEQDSKDSTYSLSSTLTLSKADYEKHKVYACEVTHQGLSSPVTKSFNRGEC

SEQ ID NO: 24 - protein, 214 aa, Artificial; identical to SEQ ID NO: 15
  Chimeric homo sapiens mus musculus

SEQ ID NO: 25 - protein, 218 aa, Artificial; identical to SEQ ID NO: 13
  Chimeric homo sapiens mus musculus

SEQ ID NO: 26 - protein, 819 aa, Artificial
  Chimeric homo sapiens mus musculus
QVQLQQSGAELVRPGSSVKISCKASGYAFSSYWMNWVKQRPGQGLEWIGQIWPGDGDTNYNGKFKGKATLTADESSSTAYMQLSSLASEDSAVYFCARRETTTVGRYYYAMDYWGQGTTVTVSSASTKGPSVFPLAPSSKSTSGGTAALGCLVKDYFPEPVTVSWNSGALTSGVHTFPAVLQSSGLYSLSSVVTVPSSSLGTQTYICNVNHKPSNTKVDKRVEPKSCDKTHTCPPCPAPELLGGPSVFLFPPKPKDTLMISRTPEVTCVVVDVSHEDPEVKFNWYVDGVEVHNAKTKPREEQYSSTYRVVSVLTVLHQDWLNGKEYKCKVSNKALPAPIEKTISKAKGQPREPQVYTLPPSREEMTKNQVSLTCLVKGFYPSDIAVEWESNGQPENNYKTTPPVLDSDGSFFLYSKLTVDKSRWQQGNVFSCSVMHEALHNHYTQKSLSLSPGGGGGSGGGGSGGGGSGQPREPQVYTLPPSREEMTKNQVSLTCLVKGFYPSDIAVEWESNGQPENNYKTTPPVLDSDGSFFLYSKLTVDKSRWQQGNVFSCSVMHEALHNHYTQKSLSLSPGSTGSEVQLQQSGPELVKPGASVKISCKTSGYTFTEYTMHWVKQSHGKSLEWIGGISPNIGGTSYNQKFKGKATLTVDKSSSTAYMELRSLTSEDSAVYYCARRGGSFDYWGQGTTLTVSSVEGGSGGSGGSGGSGGVDDIVMTQSPATLSVTPGDRVSLSCRASQSISDYLHWYQQKSHESPRLLIKYASQSISGIPSRFSGSGSGSDFTLSINSVEPEDVGVYYCQNGHSFPLTFGAGTKLELK

SEQ ID NO: 27 - protein, 218 aa, Artificial; identical to SEQ ID NO: 13
  Chimeric homo sapiens mus musculus

SEQ ID NO: 28 - protein, 819 aa, Artificial
  Chimeric homo sapiens mus musculus
QVQLQQSGAELVRPGSSVKISCKASGYAFSSYWMNWVKQRPGQGLEWIGQIWPGDGDTNYNGKFKGKATLTADESSSTAYMQLSSLASEDSAVYFCARRETTTVGRYYYAMDYWGQGTTVTVSSASTKGPSVFPLAPSSKSTSGGTAALGCLVKDYFPEPVTVSWNSGALTSGVHTFPAVLQSSGLYSLSSVVTVPSSSLGTQTYICNVNHKPSNTKVDKRVEPKSCDKTHTSPPSPAPELLGGPSVFLFPPKPKDTLMISRTPEVTCVVVDVSHEDPEVKFNWYVDGVEVHNAKTKPREEQYSSTYRVVSVLTVLHQDWLNGKEYKCKVSNKALPAPIEKTISKAKGQPREPQVYTLPPSREEMTKNQVSLTCLVKGFYPSDIAVEWESNGQPENNYKTTPPVLDSDGSFFLYSKLTVDKSRWQQGNVFSCSVMHEALHNHYTQKSLSLSPGGGGGSGGGGSGGGGSGQPREPQVYTLPPSREEMTKNQVSLTCLVKGFYPSDIAVEWESNGQPENNYKTTPPVLDSDGSFFLYSKLTVDKSRWQQGNVFSCSVMHEALHNHYTQKSLSLSPGSTGSEVQLQQSGPELVKPGASVKISCKTSGYTFTEYTMHWVKQSHGKSLEWIGGISPNIGGTSYNQKFKGKATLTVDKSSSTAYMELRSLTSEDSAVYYCARRGGSFDYWGQGTTLTVSSVEGGSGGSGGSGGSGGVDDIVMTQSPATLSVTPGDRVSLSCRASQSISDYLHWYQQKSHESPRLLIKYASQSISGIPSRFSGSGSGSDFTLSINSVEPEDVGVYYCQNGHSFPLTFGAGTKLELK

SEQ ID NO: 29 - protein, 218 aa, Artificial; identical to SEQ ID NO: 13
  Chimeric homo sapiens mus musculus

SEQ ID NO: 30 - protein, 815 aa, Artificial
  Chimeric homo sapiens mus musculus
QVQLQQSGAELVRPGSSVKISCKASGYAFSSYWMNWVKQRPGQGLEWIGQIWPGDGDTNYNGKFKGKATLTADESSSTAYMQLSSLASEDSAVYFCARRETTTVGRYYYAMDYWGQGTTVTVSSASTKGPSVFPLAPSSKSTSGGTAALGCLVKDYFPEPVTVSWNSGALTSGVHTFPAVLQSSGLYSLSSVVTVPSSSLGTQTYICNVNHKPSNTKVDKRVEPKSCGGGSSPAPELLGGPSVFLFPPKPKDTLMISRTPEVTCVVVDVSHEDPEVKFNWYVDGVEVHNAKTKPREEQYSSTYRVVSVLTVLHQDWLNGKEYKCKVSNKALPAPIEKTISKAKGQPREPQVYTLPPSREEMTKNQVSLTCLVKGFYPSDIAVEWESNGQPENNYKTTPPVLDSDGSFFLYSKLTVDKSRWQQGNVFSCSVMHEALHNHYTQKSLSLSPGGGGGSGGGGSGGGGSGQPREPQVYTLPPSREEMTKNQVSLTCLVKGFYPSDIAVEWESNGQPENNYKTTPPVLDSDGSFFLYSKLTVDKSRWQQGNVFSCSVMHEALHNHYTQKSLSLSPGSTGSEVQLQQSGPELVKPGASVKISCKTSGYTFTEYTMHWVKQSHGKSLEWIGGISPNIGGTSYNQKFKGKATLTVDKSSSTAYMELRSLTSEDSAVYYCARRGGSFDYWGQGTTLTVSSVEGGSGGSGGSGGSGGVDDIVMTQSPATLSVTPGDRVSLSCRASQSISDYLHWYQQKSHESPRLLIKYASQSISGIPSRFSGSGSGSDFTLSINSVEPEDVGVYYCQNGHSFPLTFGAGTKLELK

SEQ ID NO: 31 - protein, 819 aa, Artificial
  Chimeric homo sapiens mus musculus
DIQLTQSPASLAVSLGQRATISCKASQSVDYDGDSYLNWYQQIPGQPPKLLIYDASNLVSGIPPRFSGSGSGTDFTLNIHPVEKVDAATYHCQQSTEDPWTFGGGTKLEIKGGGGSGGGGSGGGGSQVQLQQSGAELVRPGSSVKISCKASGYAFSSYWMNWVKQRPGQGLEWIGQIWPGDGDTNYNGKFKGKATLTADESSSTAYMQLSSLASEDSAVYFCARRETTTVGRYYYAMDYWGQGTTVTVSSGGGSSAPELLGGPSVFLFPPKPKDTLMISRTPEVTCVVVDVSHEDPEVKFNWYVDGVEVHNAKTKPREEQYSSTYRVVSVLTVLHQDWLNGKEYKCKVSNKALPAPIEKTISKAKGQPREPQVYTLPPSREEMTKNQVSLTCLVKGFYPSDIAVEWESNGQPENNYKTTPPVLDSDGSFFLYSKLTVDKSRWQQGNVFSCSVMHEALHNHYTQKSLSLSPGGGGGSGGGGSGGGGSGQPREPQVYTLPPSREEMTKNQVSLTCLVKGFYPSDIAVEWESNGQPENNYKTTPPVLDSDGSFFLYSKLTVDKSRWQQGNVFSCSVMHEALHNHYTQKSLSLSPGSTGSEVQLQQSGPELVKPGASVKISCKTSGYTFTEYTMHWVKQSHGKSLEWIGGISPNIGGTSYNQKFKGKATLTVDKSSSTAYMELRSLTSEDSAVYYCARRGGSFDYWGQGTTLTVSSRTVAAPSVFIFPPSDEQLKSGTASVVCLLNNFYPREAKVQWKVDNALQSGNSQESVTEQDSKDSTYSLSSTLTLSKADYEKHKVYACEVTHQGLSSPVTKSFNRGEC

SEQ ID NO: 32 - protein, 214 aa, Artificial; identical to SEQ ID NO: 15
  Chimeric homo sapiens mus musculus

SEQ ID NO: 33 - protein, 819 aa, Artificial
  Chimeric homo sapiens mus musculus
DIQLTQSPASLAVSLGQRATISCKASQSVDYDGDSYLNWYQQIPGQPPKLLIYDASNLVSGIPPRFSGSGSGTDFTLNIHPVEKVDAATYHCQQSTEDPWTFGGGTKLEIKGGGGSGGGGSGGGGSQVQLQQSGAELVRPGSSVKISCKASGYAFSSYWMNWVKQRPGQGLEWIGQIWPGDGDTNYNGKFKGKATLTADESSSTAYMQLSSLASEDSAVYFCARRETTTVGRYYYAMDYWGQGTTVTVSSGGGSSAPELLGGPSVFLFPPKPKDTLMISRTPEVTCVVVDVSHEDPEVKFNWYVDGVEVHNAKTKPREEQYSSTYRVVSVLTVLHQDWLNGKEYKCKVSNKALPAPIEKTISKAKGQPREPQVYTLPPSREEMTKNQVSLTCLVKGFYPSDIAVEWESNGQPENNYKTTPPVLDSDGSFFLYSKLTVDKSRWQQGNVFSCSVMHEALHNHYTQKSLSLSPGGGGGSGGGGSGGGGSGQPREPQVYTLPPSREEMTKNQVSLTCLVKGFYPSDIAVEWESNGQPENNYKTTPPVLDSDGSFFLYSKLTVDKSRWQQGNVFSCSVMHEALHNHYTQKSLSLSPGSTGSEVQLQQSGPELVKPGASVKISCKTSGYTFTEYTMHWVKQSHGKSLEWIGGISPNIGGTSYNQKFKGKATLTVDKSSSTAYMELRSLTSEDSAVYYCARRGGSFDYWGQGTTLTVSSASTKGPSVFPLAPSSKSTSGGTAALGCLVKDYFPEPVTVSWNSGALTSGVHTFPAVLQSSGLYSLSSVVTVPSSSLGTQTYICNVNHKPSNTKVDKRVEPKSCDKTH

SEQ ID NO: 34 - protein, 214 aa, Artificial; identical to SEQ ID NO: 12
  Chimeric homo sapiens mus musculus

SEQ ID NO: 35 - protein, 218 aa, Artificial; identical to SEQ ID NO: 13
  Chimeric homo sapiens mus musculus

SEQ ID NO: 36 - protein, 792 aa, Artificial
  Chimeric homo sapiens mus musculus
QVQLQQSGAELVRPGSSVKISCKASGYAFSSYWMNWVKQRPGQGLEWIGQIWPGDGDTNYNGKFKGKATLTADESSSTAYMQLSSLASEDSAVYFCARRETTTVGRYYYAMDYWGQGTTVTVSSASTKGPSVFPLAPSSKSTSGGTAALGCLVKDYFPEPVTVSWNSGALTSGVHTFPAVLQSSGLYSLSSVVTVPSSSLGTQTYICNVNHKPSNTKVDKRVEPKSCDKTHTSPPSPAPELLGGPSVFLFPPKPKDTLMISRTPEVTCVVVDVSHEDPEVKFNWYVDGVEVHNAKTKPREEQYSSTYRVVSVLTVLHQDWLNGKEYKCKVSNKALPAPIEKTISKAKGQPREPQVYTLPPSREEMTKNQVSLTCLVKGFYPSDIAVEWESNGQPENNYKTTPPVLDSDGSFFLYSKLTVDKSRWQQGNVFSCSVMHEALHNHYTQKSLSLSPGGGGGSGGGGSGGGGSGQPREPQVYTLPPSREEMTKNQVSLTCLVKGFYPSDIAVEWESNGQPENNYKTTPPVLDSDGSFFLYSKLTVDKSRWQQGNVFSCSVMHEALHNHYTQKSLSLSPGSTGSDIVMTQSPATLSVTPGDRVSLSCRASQSISDYLHWYQQKSHESPRLLIKYASQSISGIPSRFSGSGSGSDFTLSINSVEPEDVGVYYCQNGHSFPLTFGAGTKLELKASTKGPSVFPLAPSSKSTSGGTAALGCLVKDYFPEPVTVSWNSGALTSGVHTFPAVLQSSGLYSLSSVVTVPSSSLGTQTYICNVNHKPSNTKVDKRVEPKSCDKTH

SEQ ID NO: 37 - protein, 223 aa, Artificial
  Chimeric homo sapiens mus musculus
EVQLQQSGPELVKPGASVKISCKTSGYTFTEYTMHWVKQSHGKSLEWIGGISPNIGGTSYNQKFKGKATLTVDKSSSTAYMELRSLTSEDSAVYYCARRGGSFDYWGQGTTLTVSSRTVAAPSVFIFPPSDEQLKSGTASVVCLLNNFYPREAKVQWKVDNALQSGNSQESVTEQDSKDSTYSLSSTLTLSKADYEKHKVYACEVTHQGLSSPVTKSFNRGEC

SEQ ID NO: 38 - protein, 445 aa, Artificial
  Chimeric homo sapiens mus musculus
DIQLTQSPASLAVSLGQRATISCKASQSVDYDGDSYLNWYQQIPGQPPKLLIYDASNLVSGIPPRFSGSGSGTDFTLNIHPVEKVDAATYHCQQSTEDPWTFGGGTKLEIKRTVAAPSVFIFPPSDEQLKSGTASVVCLLNNFYPREAKVQWKVDNALQSGNSQESVTEQDSKDSTYSLSSTLTLSKADYEKHKVYACEVTHQGLSSPVTKSFNRGECDKTHTCPPCPAPELLGGPSVFLFPPKPKDTLMISRTPEVTCVVVDVSHEDPEVKFNWYVDGVEVHNAKTKPREEQYNSTYRVVSVLTVLHQDWLNGKEYKCKVSNKALPAPIEKTISKAKGQPREPQVYTLPPSREEMTKNQVSLTCLVKGFYPSDIAVEWESNGQPENNYKTTPPVLDSDGSFFLYSKLTVDKSRWQQGNVFSCSVMHEALHNHYTQKSLSLSPGK

SEQ ID NO: 39 - protein, 680 aa, Artificial
  Chimeric homo sapiens mus musculus
QVQLQQSGAELVRPGSSVKISCKASGYAFSSYWMNWVKQRPGQGLEWIGQIWPGDGDTNYNGKFKGKATLTADESSSTAYMQLSSLASEDSAVYFCARRETTTVGRYYYAMDYWGQGTTVTVSSASTKGPSVFPLAPSSKSTSGGTAALGCLVKDYFPEPVTVSWNSGALTSGVHTFPAVLQSSGLYSLSSVVTVPSSSLGTQTYICNVNHKPSNTKVDKRVEPKSCDKTHTCPPCPAPELLGGPSVFLFPPKPKDTLMISRTPEVTCVVVDVSHEDPEVKFNWYVDGVEVHNAKTKPREEQYNSTYRVVSVLTVLHQDWLNGKEYKCKVSNKALPAPIEKTISKAKGQPREPQVYTLPPSREEMTKNQVSLTCLVKGFYPSDIAVEWESNGQPENNYKTTPPVLDSDGSFFLYSKLTVDKSRWQQGNVFSCSVMHEALHNHYTQKSLSLSPGSTGSEVQLQQSGPELVKPGASVKISCKTSGYTFTEYTMHWVKQSHGKSLEWIGGISPNIGGTSYNQKFKGKATLTVDKSSSTAYMELRSLTSEDSAVYYCARRGGSFDYWGQGTTLTVSSRTVAAPSVFIFPPSDEQLKSGTASVVCLLNNFYPREAKVQWKVDNALQSGNSQESVTEQDSKDSTYSLSSTLTLSKADYEKHKVYACEVTHQGLSSPVTKSFNRGEC

SEQ ID NO: 40 - protein, 214 aa, Artificial; identical to SEQ ID NO: 15
  Chimeric homo sapiens mus musculus

SEQ ID NO: 41 - protein, 445 aa, Artificial
  Chimeric homo sapiens mus musculus
DIQLTQSPASLAVSLGQRATISCKASQSVDYDGDSYLNWYQQIPGQPPKLLIYDASNLVSGIPPRFSGSGSGTDFTLNIHPVEKVDAATYHCQQSTEDPWTFGGGTKLEIKRTVAAPSVFIFPPSDEQLKSGTASVVCLLNNFYPREAKVQWKVDNALQSGNSQESVTEQDSKDSTYSLSSTLTLSKADYEKHKVYACEVTHQGLSSPVTKSFNRGECDKTHTCPPCPAPELLGGPSVFLFPPKPKDTLMISRTPEVTCVVVDVSHEDPEVKFNWYVDGVEVHNAKTKPREEQYSSTYRVVSVLTVLHQDWLNGKEYKCKVSNKALPAPIEKTISKAKGQPREPQVYTLPPSREEMTKNQVSLTCLVKGFYPSDIAVEWESNGQPENNYKTTPPVLDSDGSFFLYSKLTVDKSRWQQGNVFSCSVMHEALHNHYTQKSLSLSPGK

SEQ ID NO: 42 - protein, 680 aa, Artificial
  Chimeric homo sapiens mus musculus
QVQLQQSGAELVRPGSSVKISCKASGYAFSSYWMNWVKQRPGQGLEWIGQIWPGDGDTNYNGKFKGKATLTADESSSTAYMQLSSLASEDSAVYFCARRETTTVGRYYYAMDYWGQGTTVTVSSASTKGPSVFPLAPSSKSTSGGTAALGCLVKDYFPEPVTVSWNSGALTSGVHTFPAVLQSSGLYSLSSVVTVPSSSLGTQTYICNVNHKPSNTKVDKRVEPKSCDKTHTCPPCPAPELLGGPSVFLFPPKPKDTLMISRTPEVTCVVVDVSHEDPEVKFNWYVDGVEVHNAKTKPREEQYSSTYRVVSVLTVLHQDWLNGKEYKCKVSNKALPAPIEKTISKAKGQPREPQVYTLPPSREEMTKNQVSLTCLVKGFYPSDIAVEWESNGQPENNYKTTPPVLDSDGSFFLYSKLTVDKSRWQQGNVFSCSVMHEALHNHYTQKSLSLSPGSTGSEVQLQQSGPELVKPGASVKISCKTSGYTFTEYTMHWVKQSHGKSLEWIGGISPNIGGTSYNQKFKGKATLTVDKSSSTAYMELRSLTSEDSAVYYCARRGGSFDYWGQGTTLTVSSRTVAAPSVFIFPPSDEQLKSGTASVVCLLNNFYPREAKVQWKVDNALQSGNSQESVTEQDSKDSTYSLSSTLTLSKADYEKHKVYACEVTHQGLSSPVTKSFNRGEC

SEQ ID NO: 43 - protein, 214 aa, Artificial; identical to SEQ ID NO: 15
  Chimeric homo sapiens mus musculus

SEQ ID NO: 44 - protein, 445 aa, Artificial
  Chimeric homo sapiens mus musculus
DIQLTQSPASLAVSLGQRATISCKASQSVDYDGDSYLNWYQQIPGQPPKLLIYDASNLVSGIPPRFSGSGSGTDFTLNIHPVEKVDAATYHCQQSTEDPWTFGGGTKLEIKRTVAAPSVFIFPPSDEQLKSGTASVVCLLNNFYPREAKVQWKVDNALQSGNSQESVTEQDSKDSTYSLSSTLTLSKADYEKHKVYACEVTHQGLSSPVTKSFNRGESDKTHTCPPCPAPELLGGPSVFLFPPKPKDTLMISRTPEVTCVVVDVSHEDPEVKFNWYVDGVEVHNAKTKPREEQYSSTYRVVSVLTVLHQDWLNGKEYKCKVSNKALPAPIEKTISKAKGQPREPQVYTLPPSREEMTKNQVSLTCLVKGFYPSDIAVEWESNGQPENNYKTTPPVLDSDGSFFLYSKLTVDKSRWQQGNVFSCSVMHEALHNHYTQKSLSLSPGK

SEQ ID NO: 45 - protein, 680 aa, Artificial
  Chimeric homo sapiens mus musculus
QVQLQQSGAELVRPGSSVKISCKASGYAFSSYWMNWVKQRPGQGLEWIGQIWPGDGDTNYNGKFKGKATLTADESSSTAYMQLSSLASEDSAVYFCARRETTTVGRYYYAMDYWGQGTTVTVSSASTKGPSVFPLAPSSKSTSGGTAALGCLVKDYFPEPVTVSWNSGALTSGVHTFPAVLQSSGLYSLSSVVTVPSSSLGTQTYICNVNHKPSNTKVDKRVEPKSSDKTHTCPPCPAPELLGGPSVFLFPPKPKDTLMISRTPEVTCVVVDVSHEDPEVKFNWYVDGVEVHNAKTKPREEQYSSTYRVVSVLTVLHQDWLNGKEYKCKVSNKALPAPIEKTISKAKGQPREPQVYTLPPSREEMTKNQVSLTCLVKGFYPSDIAVEWESNGQPENNYKTTPPVLDSDGSFFLYSKLTVDKSRWQQGNVFSCSVMHEALHNHYTQKSLSLSPGSTGSEVQLQQSGPELVKPGASVKISCKTSGYTFTEYTMHWVKQSHGKSLEWIGGISPNIGGTSYNQKFKGKATLTVDKSSSTAYMELRSLTSEDSAVYYCARRGGSFDYWGQGTTLTVSSRTVAAPSVFIFPPSDEQLKSGTASVVCLLNNFYPREAKVQWKVDNALQSGNSQESVTEQDSKDSTYSLSSTLTLSKADYEKHKVYACEVTHQGLSSPVTKSFNRGEC

SEQ ID NO: 46 - protein, 214 aa, Artificial; identical to SEQ ID NO: 15
  Chimeric homo sapiens mus musculus

SEQ ID NO: 47 - protein, 445 aa, Artificial; identical to SEQ ID NO: 38
  Chimeric homo sapiens mus musculus

SEQ ID NO: 48 - protein, 698 aa, Artificial
  Chimeric homo sapiens mus musculus
QVQLQQSGAELVRPGSSVKISCKASGYAFSSYWMNWVKQRPGQGLEWIGQIWPGDGDTNYNGKFKGKATLTADESSSTAYMQLSSLASEDSAVYFCARRETTTVGRYYYAMDYWGQGTTVTVSSASTKGPSVFPLAPSSKSTSGGTAALGCLVKDYFPEPVTVSWNSGALTSGVHTFPAVLQSSGLYSLSSVVTVPSSSLGTQTYICNVNHKPSNTKVDKRVEPKSCDKTHTCPPCPAPELLGGPSVFLFPPKPKDTLMISRTPEVTCVVVDVSHEDPEVKFNWYVDGVEVHNAKTKPREEQYNSTYRVVSVLTVLHQDWLNGKEYKCKVSNKALPAPIEKTISKAKGQPREPQVYTLPPSREEMTKNQVSLTCLVKGFYPSDIAVEWESNGQPENNYKTTPPVLDSDGSFFLYSKLTVDKSRWQQGNVFSCSVMHEALHNHYTQKSLSLSPGSTGSEVQLQQSGPELVKPGASVKISCKTSGYTFTEYTMHWVKQSHGKSLEWIGGISPNIGGTSYNQKFKGKATLTVDKSSSTAYMELRSLTSEDSAVYYCARRGGSFDYWGQGTTLTVSSVEGGSGGSGGSGGSGGVDDIVMTQSPATLSVTPGDRVSLSCRASQSISDYLHWYQQKSHESPRLLIKYASQSISGIPSRFSGSGSGSDFTLSINSVEPEDVGVYYCQNGHSFPLTFGAGTKLELK

SEQ ID NO: 49 - protein, 444 aa, Artificial
  Chimeric homo sapiens mus musculus
IQLTQSPASLAVSLGQRATISCKASQSVDYDGDSYLNWYQQIPGQPPKLLIYDASNLVSGIPPRFSGSGSGTDFTLNIHPVEKVDAATYHCQQSTEDPWTFGGGTKLEIKRTVAAPSVFIFPPSDEQLKSGTASVVCLLNNFYPREAKVQWKVDNALQSGNSQESVTEQDSKDSTYSLSSTLTLSKADYEKHKVYACEVTHQGLSSPVTKSFNRGECDKTHTCPPCPAPELLGGPSVFLFPPKPKDTLMISRTPEVTCVVVDVSHEDPEVKFNWYVDGVEVHNAKTKPREEQYSSTYRVVSVLTVLHQDWLNGKEYKCKVSNKALPAPIEKTISKAKGQPREPQVYTLPPSREEMTKNQVSLTCLVKGFYPSDIAVEWESNGQPENNYKTTPPVLDSDGSFFLYSKLTVDKSRWQQGNVFSCSVMHEALHNHYTQKSLSLSPGK

SEQ ID NO: 50 - protein, 698 aa, Artificial
  Chimeric homo sapiens mus musculus
QVQLQQSGAELVRPGSSVKISCKASGYAFSSYWMNWVKQRPGQGLEWIGQIWPGDGDTNYNGKFKGKATLTADESSSTAYMQLSSLASEDSAVYFCARRETTTVGRYYYAMDYWGQGTTVTVSSASTKGPSVFPLAPSSKSTSGGTAALGCLVKDYFPEPVTVSWNSGALTSGVHTFPAVLQSSGLYSLSSVVTVPSSSLGTQTYICNVNHKPSNTKVDKRVEPKSCDKTHTCPPCPAPELLGGPSVFLFPPKPKDTLMISRTPEVTCVVVDVSHEDPEVKFNWYVDGVEVHNAKTKPREEQYSSTYRVVSVLTVLHQDWLNGKEYKCKVSNKALPAPIEKTISKAKGQPREPQVYTLPPSREEMTKNQVSLTCLVKGFYPSDIAVEWESNGQPENNYKTTPPVLDSDGSFFLYSKLTVDKSRWQQGNVFSCSVMHEALHNHYTQKSLSLSPGSTGSEVQLQQSGPELVKPGASVKISCKTSGYTFTEYTMHWVKQSHGKSLEWIGGISPNIGGTSYNQKFKGKATLTVDKSSSTAYMELRSLTSEDSAVYYCARRGGSFDYWGQGTTLTVSSVEGGSGGSGGSGGSGGVDDIVMTQSPATLSVTPGDRVSLSCRASQSISDYLHWYQQKSHESPRLLIKYASQSISGIPSRFSGSGSGSDFTLSINSVEPEDVGVYYCQNGHSFPLTFGAGTKLELK

SEQ ID NO: 51 - protein, 454 aa, Artificial
  Chimeric homo sapiens mus musculus
QVQLQQSGAELVRPGSSVKISCKASGYAFSSYWMNWVKQRPGQGLEWIGQIWPGDGDTNYNGKFKGKATLTADESSSTAYMQLSSLASEDSAVYFCARRETTTVGRYYYAMDYWGQGTTVTVSSASTKGPSVFPLAPSSKSTSGGTAALGCLVKDYFPEPVTVSWNSGALTSGVHTFPAVLQSSGLYSLSSVVTVPSSSLGTQTYICNVNHKPSNTKVDKRVEPKSCDKTHTCPPCPAPELLGGPSVFLFPPKPKDTLMISRTPEVTCVVVDVSHEDPEVKFNWYVDGVEVHNAKTKPREEQYSSTYRVVSVLTVLHQDWLNGKEYKCKVSNKALPAPIEKTISKAKGQPREPQVYTLPPSREEMTKNQVSLTCLVKGFYPSDIAVEWESNGQPENNYKTTPPVLDSDGSFFLYSKLTVDKSRWQQGNVFSCSVMHEALHNHYTQKSLSLSPGK

SEQ ID NO: 52 - protein, 670 aa, Artificial
  Chimeric homo sapiens mus musculus
DIQLTQSPASLAVSLGQRATISCKASQSVDYDGDSYLNWYQQIPGQPPKLLIYDASNLVSGIPPRFSGSGSGTDFTLNIHPVEKVDAATYHCQQSTEDPWTFGGGTKLEIKRTVAAPSVFIFPPSDEQLKSGTASVVCLLNNFYPREAKVQWKVDNALQSGNSQESVTEQDSKDSTYSLSSTLTLSKADYEKHKVYACEVTHQGLSSPVTKSFNRGECDKTHTCPPCPAPELLGGPSVFLFPPKPKDTLMISRTPEVTCVVVDVSHEDPEVKFNWYVDGVEVHNAKTKPREEQSSTYRVVSVLTVLHQDWLNGKEYKCKVSNKALPAPIEKTISKAKGQPREPQVYTLPPSREEMTKNQVSLTCLVKGFYPSDIAVEWESNGQPENNYKTTPPVLDSDGSFFLYSKLTVDKSRWQQGNVFSCSVMHEALHNHYTQKSLSLSPGSTGSEVQLQQSGPELVKPGASVKISCKTSGYTFTEYTMHWVKQSHGKSLEWIGGISPNIGGTSYNQKFKGKATLTVDKSSSTAYMELRSLTSEDSAVYYCARRGGSFDYWGQGTTLTVSSRTVAAPSVFIFPPSDEQLKSGTASVVCLLNNFYPREAKVQWKVDNALQSGNSQESVTEQDSKDSTYSLSSTLTLSKADYEKHKVYACEVTHQGLSSPVTKSFNRGEC

SEQ ID NO: 53 - protein, 214 aa, Artificial; identical to SEQ ID NO: 15
  Chimeric homo sapiens mus musculus

SEQ ID NO: 54 - protein, 445 aa, Artificial; identical to SEQ ID NO: 41
  Chimeric homo sapiens mus musculus

SEQ ID NO: 55 - protein, 671 aa, Artificial
  Chimeric homo sapiens mus musculus
QVQLQQSGAELVRPGSSVKISCKASGYAFSSYWMNWVKQRPGQGLEWIGQIWPGDGDTNYNGKFKGKATLTADESSSTAYMQLSSLASEDSAVYFCARRETTTVGRYYYAMDYWGQGTTVTVSSASTKGPSVFPLAPSSKSTSGGTAALGCLVKDYFPEPVTVSWNSGALTSGVHTFPAVLQSSGLYSLSSVVTVPSSSLGTQTYICNVNHKPSNTKVDKRVEPKSCDKTHTCPPCPAPELLGGPSVFLFPPKPKDTLMISRTPEVTCVVVDVSHEDPEVKFNWYVDGVEVHNAKTKPREEQYSSTYRVVSVLTVLHQDWLNGKEYKCKVSNKALPAPIEKTISKAKGQPREPQVYTLPPSREEMTKNQVSLTCLVKGFYPSDIAVEWESNGQPENNYKTTPPVLDSDGSFFLYSKLTVDKSRWQQGNVFSCSVMHEALHNHYTQKSLSLSPGSTGSDIVMTQSPATLSVTPGDRVSLSCRASQSISDYLHWYQQKSHESPRLLIKYASQSISGIPSRFSGSGSGSDFTLSINSVEPEDVGVYYCQNGHSFPLTFGAGTKLELKASTKGPSVFPLAPSSKSTSGGTAALGCLVKDYFPEPVTVSWNSGALTSGVHTFPAVLQSSGLYSLSSVVTVPSSSLGTQTYICNVNHKPSNTKVDKRVEPKSCDKTH

SEQ ID NO: 56 - protein, 223 aa, Artificial; identical to SEQ ID NO: 37
  Chimeric homo sapiens mus musculus